European Patent Specification EP 3 990 667 B1, published January 31, 2024. Title: METHODS AND REAGENTS FOR THE SPECIFIC AND SENSITIVE DETECTION OF SARS-CoV-2. Applicant: INSTITUT PASTEUR. The sequence listing filed with the application follows.

SEQUENCE LISTING (46 sequences)

SEQ ID NO: 1 - DNA, 18 bp, artificial sequence
  synthetic oligonucleotide (forward primer nCoV_IP2-12669Fw)
atgagcttagtcctgttg

SEQ ID NO: 2 - DNA, 18 bp, artificial sequence
  synthetic oligonucleotide (reverse primer nCoV_IP2-12759Rv)
ctccctttgttgtgttgt

SEQ ID NO: 3 - DNA, 21 bp, artificial sequence
  synthetic oligonucleotide (probe nCoV_IP2-12696bProbe(+))
agatgtcttgtgctgccggta

SEQ ID NO: 4 - DNA, 19 bp, artificial sequence
  synthetic oligonucleotide (forward primer nCoV_IP4-14059Fw)
ggtaactggtatgatttcg

SEQ ID NO: 5 - DNA, 20 bp, artificial sequence
  synthetic oligonucleotide (reverse primer nCoV_IP4-14146Rv)
ctggtcaaggttaatatagg

SEQ ID NO: 6 - DNA, 19 bp, artificial sequence
  synthetic oligonucleotide (probe nCoV_IP4-14084Probe(+))
tcatacaaaccacgccagg

SEQ ID NO: 7 - DNA, 26 bp, artificial sequence
  synthetic oligonucleotide (forward primer E_Sarbeco_F1)
acaggtacgttaatagttaatagcgt

SEQ ID NO: 8 - DNA, 22 bp, artificial sequence
  synthetic oligonucleotide (reverse primer E_Sarbeco_R2)
atattgcagcagtacgcacaca

SEQ ID NO: 9 - DNA, 26 bp, artificial sequence
  synthetic oligonucleotide (probe E_Sarbeco_P1)
acactagccatccttactgcgcttcg

SEQ ID NO: 10 - DNA, 18 bp, artificial sequence
  synthetic oligonucleotide (target sequence)
caacaggactaagctcat

SEQ ID NO: 11 - DNA, 18 bp, artificial sequence
  synthetic oligonucleotide (target sequence)
acaacacaacaaagggag

SEQ ID NO: 12 - DNA, 21 bp, artificial sequence
  synthetic oligonucleotide (target sequence)
taccggcagcacaagacatct

SEQ ID NO: 13 - DNA, 19 bp, artificial sequence
  synthetic oligonucleotide (target sequence)
cgaaatcataccagttacc

SEQ ID NO: 14 - DNA, 20 bp, artificial sequence
  synthetic oligonucleotide (target sequence)
cctatattaaccttgaccag

SEQ ID NO: 15 - DNA, 19 bp, artificial sequence
  synthetic oligonucleotide (target sequence)
cctggcgtggtttgtatga

SEQ ID NO: 16 - DNA, 108 bp, artificial sequence
  synthetic polynucleotide (nCoV_IP2 amplification product)
atgagcttagtcctgttgcactacgacagatgtcttgtgctgccggtactacacaaactgcttgcactgatgacaatgcgttagcttactacaacacaacaaagggag

SEQ ID NO: 17 - DNA, 107 bp, artificial sequence
  synthetic polynucleotide (nCoV_IP4 amplification product)
ggtaactggtatgatttcggtgatttcatacaaaccacgccaggtagtggagttcctgttgtagattcttattattcattgttaatgcctatattaaccttgaccag

SEQ ID NO: 18 - DNA, 113 bp, artificial sequence
  synthetic polynucleotide (E_Sarbeco amplification product)
acaggtacgttaatagttaatagcgtacttctttttcttgctttcgtggtattcttgctagttacactagccatccttactgcgcttcgattgtgtgcgtactgctgcaatat

SEQ ID NO: 19 - DNA, 29788 bp, SARS-CoV-2
aggtaacaaaccaaccaactttcgatctcttgtagatctgttctctaaacgaactttaaaatctgtgtggctgtcactcggctgcatgcttagtgcactcacgcagtataattaataactaattactgtcgttgacaggacacgagtaactcgtctatcttctgcaggctgcttacggtttcgtccgtgttgcagccgatcatcagcacatctaggtttcgtccgggtgtgaccgaaaggtaagatggagagccttgtccctggtttcaacgagaaaacacacgtccaactcagtttgcctgttttacaggttcgcgacgtgctcgtacgtggctttggagactccgtggaggaggtcttatcagaggcacgtcaacatcttaaagatggcacttgtggcttagtagaagttgaaaaaggcgttttgcctcaacttgaacagccctatgtgttcatcaaacgttcggatgctcgaactgcacctcatggtcatgttatggttgagctggtagcagaactcgaaggcattcagtacggtcgtagtggtgagacacttggtgtccttgtccctcatgtgggcgaaataccagtggcttaccgcaaggttcttcttcgtaagaacggtaataaaggagctggtggccatggttacggcgccgatctaaagtcatttgacttaggcgacgagcttggcactgatccttatgaagattttcaagaaaactggaacactaaacatagcagtggtgttacccgtgaactcatgcgtgagcttaacggaggggcatacactcgctatgtcgataacaacttctgtggccctgatggctaccctcttgagtgcattaaagaccttctagcacgtgctggtaaagcttcatgcactttgtccgaacaactggactttattgacactaagaggggtgtatactgctgccgtgaacatgagcatgaaattgcttggtacacggaacgttctgaaaagagctatgaattgcagacaccttttgaaattaaattggcaaagaaatttgacaccttcaatggggaatgtccaaattttgtatttcccttaaattccataatcaagactattcaaccaagggttgaaaagaaaaagcttgatggctttatgggtagaattcgatctgtctatccagttgcgtcaccaaatgaatgcaaccaaatgtgcctttcaactctcatgaagtgtgatcattgtggtgaaacttcatggcagacgggcgattttgttaaagccacttgcgaattttgtggcactgagaatttgactaaagaaggtgccactacttgtggttacttaccccaaaatgctgttgttaaaatttattgtccagcatgtcacaattcagaagtaggacctgagcatagtcttgccgaataccataatgaatctggcttgaaaaccattcttcgtaagggtggtcgcactattgcctttggaggctgtgtgttctcttatgttggttgccataacaagtgtgcctattgggttccacgtgctagcgctaacataggttgtaaccatacaggtgttgttggagaaggttccgaaggtcttaatgacaaccttcttgaaatactccaaaaagagaaagtcaacatcaatattgttggtgactttaaacttaatgaagagatcgccattattttggcatctttttctgcttccacaagtgcttttgtggaaactgtgaaaggtttggattataaagcattcaaacaaattgttgaatcctgtggtaattttaaagttacaaaaggaaaagctaaaaaaggtgcctggaatattggtgaacagaaatcaatactgagtcctctttatgcatttgcatcagaggctgctcgtgttgtacgatcaattttctcccgcactcttgaaactgctcaaaattctgtgcgtgttttacagaaggccgctataacaatactagatggaatttcacagtattcactgagactcattgatgctatgatgttcacatctgatttggctactaacaatctagttgtaatggcctacattacaggtggtgttgttcagttgacttcgcagtggctaactaacatctttggcactgtttatgaaaaactcaaacccgtccttgattggcttgaagagaagtttaaggaaggtgtagagtttcttagagacggttgggaaattgttaaatttatctcaacctgtgcttgtgaaattgtcggtggacaaattgtcacctgtgcaaaggaaattaaggagagtgttcagacattctttaagcttgtaaataaatttttggctttgtgtgctgactctatcattattggtggagctaaacttaaagccttgaatttaggtgaaacatttgtcacgcactcaaagggattgtacagaaagtgtgttaaatccagagaagaaactggcctactcatgcctctaaaagccccaaaagaaattatcttcttagagggagaaacacttcccacagaagtgttaacagaggaagttgtcttgaaaactggtgatttacaaccattagaacaacctactagtgaagctgttgaagctccattggttggtacaccagtttgtattaacgggcttatgttgctcgaaatcaaagacacagaaaagtactgtgcccttgcacctaatatgatggtaacaaacaataccttcacactcaaaggcggtgcaccaacaaaggttacttttggtgatgacactgtgatagaagtgcaaggttacaagagtgtgaatatcacttttgaacttgatgaaaggattgataaagtacttaatgagaagtgctctgcctatacagttgaactcggtacagaagtaaatgagttcgcctgtgttgtggcagatgctgtcataaaaactttgcaaccagtatctgaattacttacaccactgggcattgatttagatgagtggagtatggctacatactacttatttgatgagtctggtgagtttaaattggcttcacatatgtattgttctttctaccctccagatgaggatgaagaagaaggtgattgtgaagaagaagagtttgagccatcaactcaatatgagtatggtactgaagatgattaccaaggtaaacctttggaatttggtgccacttctgctgctcttcaacctgaagaagagcaagaagaagattggttagatgatgatagtcaacaaactgttggtcaacaagacggcagtgaggacaatcagacaactactattcaaacaattgttgaggttcaacctcaattagagatggaacttacaccagttgttcagactattgaagtgaatagttttagtggttatttaaaacttactgacaatgtatacattaaaaatgcagacattgtggaagaagctaaaaaggtaaaaccaacagtggttgttaatgcagccaatgtttaccttaaacatggaggaggtgttgcaggagccttaaataaggctactaacaatgccatgcaagttgaatctgatgattacatagctactaatggaccacttaaagtgggtggtagttgtgttttaagcggacacaatcttgctaaacactgtcttcatgttgtcggcccaaatgttaacaaaggtgaagacattcaacttcttaagagtgcttatgaaaattttaatcagcacgaagttctacttgcaccattattatcagctggtatttttggtgctgaccctatacattctttaagagtttgtgtagatactgttcgcacaaatgtctacttagctgtctttgataaaaatctctatgacaaacttgtttcaagctttttggaaatgaagagtgaaaagcaagttgaacaaaagatcgctgagattcctaaagaggaagttaagccatttataactgaaagtaaaccttcagttgaacagagaaaacaagatgataagaaaatcaaagcttgtgttgaagaagttacaacaactctggaagaaactaagttcctcacagaaaacttgttactttatattgacattaatggcaatcttcatccagattctgccactcttgttagtgacattgacatcactttcttaaagaaagatgctccatatatagtgggtgatgttgttcaagagggtgttttaactgctgtggttatacctactaaaaaggctggtggcactactgaaatgctagcgaaagctttgagaaaagtgccaacagacaattatataaccacttacccgggtcagggtttaaatggttacactgtagaggaggcaaagacagtgcttaaaaagtgtaaaagtgccttttacattctaccatctattatctctaatgagaagcaagaaattcttggaactgtttcttggaatttgcgagaaatgcttgcacatgcagaagaaacacgcaaattaatgcctgtctgtgtggaaactaaagccatagtttcaactatacagcgtaaatataagggtattaaaatacaagagggtgtggttgattatggtgctagattttacttttacaccagtaaaacaactgtagcgtcacttatcaacacacttaacgatctaaatgaaactcttgttacaatgccacttggctatgtaacacatggcttaaatttggaagaagctgctcggtatatgagatctctcaaagtgccagctacagtttctgtttcttcacctgatgctgttacagcgtataatggttatcttacttcttcttctaaaacacctgaagaacattttattgaaaccatctcacttgctggttcctataaagattggtcctattctggacaatctacacaactaggtatagaatttcttaagagaggtgataaaagtgtatattacactagtaatcctaccacattccacctagatggtgaagttatcacctttgacaatcttaagacacttctttctttgagagaagtgaggactattaaggtgtttacaacagtagacaacattaacctccacacgcaagttgtggacatgtcaatgacatatggacaacagtttggtccaacttatttggatggagctgatgttactaaaataaaacctcataattcacatgaaggtaaaacattttatgttttacctaatgatgacactctacgtgttgaggcttttgagtactaccatacaactgatcctagttttctgggtaggtacatgtcagcattaaatcacactaaaaagtggaaatacccacaagttaatggtttaacttctattaaatgggcagataacaactgttatcttgccactgcattgttaacactccaacaaatagagttgaagtttaatccacctgctctacaagatgcttattacagagcaagggctggtgaagctgctaacttttgtgcacttatcttagcctactgtaataagacagtaggtgagttaggtgatgttagagaaacaatgagttacttgtttcaacatgccaatttagattcttgcaaaagagtcttgaacgtggtgtgtaaaacttgtggacaacagcagacaacccttaagggtgtagaagctgttatgtacatgggcacactttcttatgaacaatttaagaaaggtgttcagataccttgtacgtgtggtaaacaagctacaaaatatctagtacaacaggagtcaccttttgttatgatgtcagcaccacctgctcagtatgaacttaagcatggtacatttacttgtgctagtgagtacactggtaattaccagtgtggtcactataaacatataacttctaaagaaactttgtattgcatagacggtgctttacttacaaagtcctcagaatacaaaggtcctattacggatgttttctacaaagaaaacagttacacaacaaccataaaaccagttacttataaattggatggtgttgtttgtacagaaattgaccctaagttggacaattattataagaaataccattcttatttcacagagcaaccaattgatcttgtaccaaaccaaccatatccaaacgcaagcttcgataattttaagtttgtatgtgataatatcaaatttgctgatgatttaaaccagttaactggttataagaaacctgcttcaagagagcttaaagttacatttttccctgacttaaatggtgatgtggtggctattgattataaacactacacaccctcttttaagaaaggagctaaattgttacataaacctattgtttggcatgttaacaatgcaactaataaagccacgtataaaccaaatacctggtgtatacgttgtctttggagcacaaaaccagttgaaacatcaaattcgtttgatgtactgaagtcagaggacgcgcagggaatggataatcttgcctgcgaagatctaaaaccagtctctgaagaagtagtggaaaatcctaccatacagaaagacgttcttgagtgtaatgtgaaaactaccgaagttgtaggagacattatacttaaaccagcaaataatagtttaaaaattacagaagaggttggccacacagatctaatggctgcttatgtagacaattctagtcttactattaagaaacctaatgaattatctagagtattaggtttgaaaacccttgctactcatggtttagctgctgttaatagtgtcccttgggatactatagctaattatgctaagccttttcttaacaaagttgttagtacaactactaacatagttacacggtgtttaaaccgtgtttgtactaattatatgccttatttctttactttattgctacaattgtgtacttttactagaagtacaaattctagaattaaagcatctatgccgactactatagcaaagaatactgttaagagtgtcagtaaattttgtctagaggcttcatttaattatttgaagtcacctaatttttctaaactgataaatattataatttggtttttactattaagtgtttgcctaggttctttaatctactcaaccgctgctttaggtgttttaatgtctaatttaggcatgccttcttactgtactggttacagagaaggctatttgaactctactaatgtcactattgcaacctactgtactggttctataccttgtagtgtttgtcttagtggtttagattctttagacacctatccttctttagaaactatacaaattaccatttcatcttttaaatgggatttaactgcttttggcttagttgcagagtggtttttggcatatattcttttcactaggtttttctatgtacttggattggctgcaatcatgcaattgtttttcagctattttgcagtacattttattagtaattcttggcttatgtggttaataattaatcttgtacaaatggccctgatttcagctatggttagaatgtacatcttctttgcatcattttattatgtatggaaaagttatgtgcatgttgtagacggttgtaattcatcaacttgtatgatgtgttacaaacgtaatagagcaacaagagtcgaatgtacaactattgttaatggtgttagaaggtccttttatgtctatgctaatggaggtaaaggcttttgcaaactacacaattggaattgtgttaattgtgatacattctgtgctggtagtacatttattagtgatgaagttgcgagagacttgtcactacagtttaaaagaccaataaatcctactgaccagtcttcttacatcgttgatagtgttacagtgaagaatggttccatccatctttactttgataaagctggtcaaaagacttatgaaagacattctctctctcattttgttaacttagacaacctgagagctaataacactaaaggttcattgcctattaatgttatagtttttgatggtaaatcaaaatgtgaagaatcatctgcaaaatcagcgtctgtttactacagtcagcttatgtgtcaacctatactgttactagatcaggcattagtgtctgatgttggtgatagtgcggaagttgcagttaaaatgtttgatgcttacgttaatacgttttcatcaacttttaacgtaccaatggaaaaactcaaaacactagttgcaactgcagaagctgaacttgcaaagaatgtgtccttagacaatgtcttatctacttttatttcagcagctcggcaagggtttgttgattcagatgtagaaactaaagatgttgttgaatgtcttaaattgtcacatcaatctgacatagaagttactggcgatagttgtaataactatatgctcacctataacaaagttgaaaacatgacaccccgtgaccttggtgcttgtattgactgtagtgcgcgtcatattaatgcgcaggtagcaaaaagtcacaacattgctttgatatggaacgttaaagatttcatgtcattgtctgaacaactacgaaaacaaatacgtagtgctgctaaaaagaataacttaccttttaagttgacatgtgcaactactagacaagttgttaatgttgtaacaacaaagatagcacttaagggtggtaaaattgttaataattggttgaagcagttaattaaagttacacttgtgttcctttttgttgctgctattttctatttaataacacctgttcatgtcatgtctaaacatactgacttttcaagtgaaatcataggatacaaggctattgatggtggtgtcactcgtgacatagcatctacagatacttgttttgctaacaaacatgctgattttgacacatggtttagccagcgtggtggtagttatactaatgacaaagcttgcccattgattgctgcagtcataacaagagaagtgggttttgtcgtgcctggtttgcctggcacgatattacgcacaactaatggtgactttttgcatttcttacctagagtttttagtgcagttggtaacatctgttacacaccatcaaaacttatagagtacactgactttgcaacatcagcttgtgttttggctgctgaatgtacaatttttaaagatgcttctggtaagccagtaccatattgttatgataccaatgtactagaaggttctgttgcttatgaaagtttacgccctgacacacgttatgtgctcatggatggctctattattcaatttcctaacacctaccttgaaggttctgttagagtggtaacaacttttgattctgagtactgtaggcacggcacttgtgaaagatcagaagctggtgtttgtgtatctactagtggtagatgggtacttaacaatgattattacagatctttaccaggagttttctgtggtgtagatgctgtaaatttacttactaatatgtttacaccactaattcaacctattggtgctttggacatatcagcatctatagtagctggtggtattgtagctatcgtagtaacatgccttgcctactattttatgaggtttagaagagcttttggtgaatacagtcatgtagttgcctttaatactttactattccttatgtcattcactgtactctgtttaacaccagtttactcattcttacctggtgtttattctgttatttacttgtacttgacattttatcttactaatgatgtttcttttttagcacatattcagtggatggttatgttcacacctttagtacctttctggataacaattgcttatatcatttgtatttccacaaagcatttctattggttctttagtaattacctaaagagacgtgtagtctttaatggtgtttcctttagtacttttgaagaagctgcgctgtgcacctttttgttaaataaagaaatgtatctaaagttgcgtagtgatgtgctattacctcttacgcaatataatagatacttagctctttataataagtacaagtattttagtggagcaatggatacaactagctacagagaagctgcttgttgtcatctcgcaaaggctctcaatgacttcagtaactcaggttctgatgttctttaccaaccaccacaaacctctatcacctcagctgttttgcagagtggttttagaaaaatggcattcccatctggtaaagttgagggttgtatggtacaagtaacttgtggtacaactacacttaacggtctttggcttgatgacgtagtttactgtccaagacatgtgatctgcacctctgaagacatgcttaaccctaattatgaagatttactcattcgtaagtctaatcataatttcttggtacaggctggtaatgttcaactcagggttattggacattctatgcaaaattgtgtacttaagcttaaggttgatacagccaatcctaagacacctaagtataagtttgttcgcattcaaccaggacagactttttcagtgttagcttgttacaatggttcaccatctggtgtttaccaatgtgctatgaggcccaatttcactattaagggttcattccttaatggttcatgtggtagtgttggttttaacatagattatgactgtgtctctttttgttacatgcaccatatggaattaccaactggagttcatgctggcacagacttagaaggtaacttttatggaccttttgttgacaggcaaacagcacaagcagctggtacggacacaactattacagttaatgttttagcttggttgtacgctgctgttataaatggagacaggtggtttctcaatcgatttaccacaactcttaatgactttaaccttgtggctatgaagtacaattatgaacctctaacacaagaccatgttgacatactaggacctctttctgctcaaactggaattgccgttttagatatgtgtgcttcattaaaagaattactgcaaaatggtatgaatggacgtaccatattgggtagtgctttattagaagatgaatttacaccttttgatgttgttagacaatgctcaggtgttactttccaaagtgcagtgaaaagaacaatcaagggtacacaccactggttgttactcacaattttgacttcacttttagttttagtccagagtactcaatggtctttgttcttttttttgtatgaaaatgcctttttaccttttgctatgggtattattgctatgtctgcttttgcaatgatgtttgtcaaacataagcatgcatttctctgtttgtttttgttaccttctcttgccactgtagcttattttaatatggtctatatgcctgctagttgggtgatgcgtattatgacatggttggatatggttgatactagtttgtctggttttaagctaaaagactgtgttatgtatgcatcagctgtagtgttactaatccttatgacagcaagaactgtgtatgatgatggtgctaggagagtgtggacacttatgaatgtcttgacactcgtttataaagtttattatggtaatgctttagatcaagccatttccatgtgggctcttataatctctgttacttctaactactcaggtgtagttacaactgtcatgtttttggccagaggtattgtttttatgtgtgttgagtattgccctattttcttcataactggtaatacacttcagtgtataatgctagtttattgtttcttaggctatttttgtacttgttactttggcctcttttgtttactcaaccgctactttagactgactcttggtgtttatgattacttagtttctacacaggagtttagatatatgaattcacagggactactcccacccaagaatagcatagatgccttcaaactcaacattaaattgttgggtgttggtggcaaaccttgtatcaaagtagccactgtacagtctaaaatgtcagatgtaaagtgcacatcagtagtcttactctcagttttgcaacaactcagagtagaatcatcatctaaattgtgggctcaatgtgtccagttacacaatgacattctcttagctaaagatactactgaagcctttgaaaaaatggtttcactactttctgttttgctttccatgcagggtgctgtagacataaacaagctttgtgaagaaatgctggacaacagggcaaccttacaagctatagcctcagagtttagttcccttccatcatatgcagcttttgctactgctcaagaagcttatgagcaggctgttgctaatggtgattctgaagttgttcttaaaaagttgaagaagtctttgaatgtggctaaatctgaatttgaccgtgatgcagccatgcaacgtaagttggaaaagatggctgatcaagctatgacccaaatgtataaacaggctagatctgaggacaagagggcaaaagttactagtgctatgcagacaatgcttttcactatgcttagaaagttggataatgatgcactcaacaacattatcaacaatgcaagagatggttgtgttcccttgaacataatacctcttacaacagcagccaaactaatggttgtcataccagactataacacatataaaaatacgtgtgatggtacaacatttacttatgcatcagcattgtgggaaatccaacaggttgtagatgcagatagtaaaattgttcaacttagtgaaattagtatggacaattcacctaatttagcatggcctcttattgtaacagctttaagggccaattctgctgtcaaattacagaataatgagcttagtcctgttgcactacgacagatgtcttgtgctgccggtactacacaaactgcttgcactgatgacaatgcgttagcttactacaacacaacaaagggaggtaggtttgtacttgcactgttatccgatttacaggatttgaaatgggctagattccctaagagtgatggaactggtactatctatacagaactggaaccaccttgtaggtttgttacagacacacctaaaggtcctaaagtgaagtatttatactttattaaaggattaaacaacctaaatagaggtatggtacttggtagtttagctgccacagtacgtctacaagctggtaatgcaacagaagtgcctgccaattcaactgtattatctttctgtgcttttgctgtagatgctgctaaagcttacaaagattatctagctagtgggggacaaccaatcactaattgtgttaagatgttgtgtacacacactggtactggtcaggcaataacagttacaccggaagccaatatggatcaagaatcctttggtggtgcatcgtgttgtctgtactgccgttgccacatagatcatccaaatcctaaaggattttgtgacttaaaaggtaagtatgtacaaatacctacaacttgtgctaatgaccctgtgggttttacacttaaaaacacagtctgtaccgtctgcggtatgtggaaaggttatggctgtagttgtgatcaactccgcgaacccatgcttcagtcagctgatgcacaatcgtttttaaacgggtttgcggtgtaagtgcagcccgtcttacaccgtgcggcacaggcactagtactgatgtcgtatacagggcttttgacatctacaatgataaagtagctggttttgctaaattcctaaaaactaattgttgtcgcttccaagaaaaggacgaagatgacaatttaattgattcttactttgtagttaagagacacactttctctaactaccaacatgaagaaacaatttataatttacttaaggattgtccagctgttgctaaacatgacttctttaagtttagaatagacggtgacatggtaccacatatatcacgtcaacgtcttactaaatacacaatggcagacctcgtctatgctttaaggcattttgatgaaggtaattgtgacacattaaaagaaatacttgtcacatacaattgttgtgatgatgattatttcaataaaaaggactggtatgattttgtagaaaacccagatatattacgcgtatacgccaacttaggtgaacgtgtacgccaagctttgttaaaaacagtacaattctgtgatgccatgcgaaatgctggtattgttggtgtactgacattagataatcaagatctcaatggtaactggtatgatttcggtgatttcatacaaaccacgccaggtagtggagttcctgttgtagattcttattattcattgttaatgcctatattaaccttgaccagggctttaactgcagagtcacatgttgacactgacttaacaaagccttacattaagtgggatttgttaaaatatgacttcacggaagagaggttaaaactctttgaccgttattttaaatattgggatcagacataccacccaaattgtgttaactgtttggatgacagatgcattctgcattgtgcaaactttaatgttttattctctacagtgttcccacctacaagttttggaccactagtgagaaaaatatttgttgatggtgttccatttgtagtttcaactggataccacttcagagagctaggtgttgtacataatcaggatgtaaacttacatagctctagacttagttttaaggaattacttgtgtatgctgctgaccctgctatgcacgctgcttctggtaatctattactagataaacgcactacgtgcttttcagtagctgcacttactaacaatgttgcttttcaaactgtcaaacccggtaattttaacaaagacttctatgactttgctgtgtctaagggtttctttaaggaaggaagttctgttgaattaaaacacttcttctttgctcaggatggtaatgctgctatcagcgattatgactactatcgttataatctaccaacaatgtgtgatatcagacaactactatttgtagttgaagttgttgataagtactttgattgttacgatggtggctgtattaatgctaaccaagtcatcgtcaacaacctagacaaatcagctggttttccatttaataaatggggtaaggctagactttattatgattcaatgagttatgaggatcaagatgcacttttcgcatatacaaaacgtaatgtcatccctactataactcaaatgaatcttaagtatgccattagtgcaaagaatagagctcgcaccgtagctggtgtctctatctgtagtactatgaccaatagacagtttcatcaaaaattattgaaatcaatagccgccactagaggagctactgtagtaattggaacaagcaaattctatggtggttggcacaacatgttaaaaactgtttatagtgatgtagaaaaccctcaccttatgggttgggattatcctaaatgtgatagagccatgcctaacatgcttagaattatggcctcacttgttcttgctcgcaaacatacaacgtgttgtagcttgtcacaccgtttctatagattagctaatgagtgtgctcaagtattgagtgaaatggtcatgtgtggcggttcactatatgttaaaccaggtggaacctcatcaggagatgccacaactgcttatgctaatagtgtttttaacatttgtcaagctgtcacggccaatgttaatgcacttttatctactgatggtaacaaaattgccgataagtatgtccgcaatttacaacacagactttatgagtgtctctatagaaatagagatgttgacacagactttgtgaatgagttttacgcatatttgcgtaaacatttctcaatgatgatactctctgacgatgctgttgtgtgtttcaatagcacttatgcatctcaaggtctagtggctagcataaagaactttaagtcagttctttattatcaaaacaatgtttttatgtctgaagcaaaatgttggactgagactgaccttactaaaggacctcatgaattttgctctcaacatacaatgctagttaaacagggtgatgattatgtgtaccttccttacccagatccatcaagaatcctaggggccggctgttttgtagatgatatcgtaaaaacagatggtacacttatgattgaacggttcgtgtctttagctatagatgcttacccacttactaaacatcctaatcaggagtatgctgatgtctttcatttgtacttacaatacataagaaagctacatgatgagttaacaggacacatgttagacatgtattctgttatgcttactaatgataacacttcaaggtattgggaacctgagttttatgaggctatgtacacaccgcatacagtcttacaggctgttggggcttgtgttctttgcaattcacagacttcattaagatgtggtgcttgcatacgtagaccattcttatgttgtaaatgctgttacgaccatgtcatatcaacatcacataaattagtcttgtctgttaatccgtatgtttgcaatgctccaggttgtgatgtcacagatgtgactcaactttacttaggaggtatgagctattattgtaaatcacataaaccacccattagttttccattgtgtgctaatggacaagtttttggtttatataaaaatacatgtgttggtagcgataatgttactgactttaatgcaattgcaacatgtgactggacaaatgctggtgattacattttagctaacacctgtactgaaagactcaagctttttgcagcagaaacgctcaaagctactgaggagacatttaaactgtcttatggtattgctactgtacgtgaagtgctgtctgacagagaattacatctttcatgggaagttggtaaacctagaccaccacttaaccgaaattatgtctttactggttatcgtgtaactaaaaacagtaaagtacaaataggagagtacacctttgaaaaaggtgactatggtgatgctgttgtttaccgaggtacaacaacttacaaattaaatgttggtgattattttgtgctgacatcacatacagtaatgccattaagtgcacctacactagtgccacaagagcactatgttagaattactggcttatacccaacactcaatatctcagatgagttttctagcaatgttgcaaattatcaaaaggttggtatgcaaaagtattctacactccagggaccacctggtactggtaagagtcattttgctattggcctagctctctactacccttctgctcgcatagtgtatacagcttgctctcatgccgctgttgatgcactatgtgagaaggcattaaaatatttgcctatagataaatgtagtagaattatacctgcacgtgctcgtgtagagtgttttgataaattcaaagtgaattcaacattagaacagtatgtcttttgtactgtaaatgcattgcctgagacgacagcagatatagttgtctttgatgaaatttcaatggccacaaattatgatttgagtgttgtcaatgccagattacgtgctaagcactatgtgtacattagcgaccctgctcaattacctgcaccacgcacattgctaactaagggcacactagaaccagaatatttcaattcagtgtgtagacttatgaaaactataggtccagacatgttcctcggaacttgtcggcgttgtcctgctgaaattgttgacactgtgagtgctttggtttatgataataagcttaaagcacataaagacaaatcagctcaatgctttaaaatgttttataagggtgttatcacgcatgatgtttcatctgcaattaacaggccacaaataggcgtggtaagagaattccttacacgtaaccctgcttggagaaaagctgtctttatttcaccttataattcacagaatgctgtagcctcaaagattttgggactaccaactcaaactgttgattcatcacagggctcagaatatgactatgtcatattcactcaaaccactgaaacagctcactcttgtaatgtaaacagatttaatgttgctattaccagagcaaaagtaggcatactttgcataatgtctgatagagacctttatgacaagttgcaatttacaagtcttgaaattccacgtaggaatgtggcaactttacaagctgaaaatgtaacaggactctttaaagattgtagtaaggtaatcactgggttacatcctacacaggcacctacacacctcagtgttgacactaaattcaaaactgaaggtttatgtgttgacatacctggcatacctaaggacatgacctatagaagactcatctctatgatgggttttaaaatgaattatcaagttaatggttaccctaacatgtttatcacccgcgaagaagctataagacatgtacgtgcatggattggcttcgatgtcgaggggtgtcatgctactagagaagctgttggtaccaatttacctttacagctaggtttttctacaggtgttaacctagttgctgtacctacaggttatgttgatacacctaataatacagatttttccagagttagtgctaaaccaccgcctggagatcaatttaaacaccttataccacttatgtacaaaggacttccttggaatgtagtgcgtataaagattgtacaaatgttaagtgacacacttaaaaatctctctgacagagtcgtatttgtcttatgggcacatggctttgagttgacatctatgaagtattttgtgaaaataggacctgagcgcacctgttgtctatgtgatagacgtgccacatgcttttccactgcttcagacacttatgcctgttggcatcattctattggatttgattacgtctataatccgtttatgattgatgttcaacaatggggttttacaggtaacctacaaagcaaccatgatctgtattgtcaagtccatggtaatgcacatgtagctagttgtgatgcaatcatgactaggtgtctagctgtccacgagtgctttgttaagcgtgttgactggactattgaatatcctataattggtgatgaactgaagattaatgcggcttgtagaaaggttcaacacatggttgttaaagctgcattattagcagacaaattcccagttcttcacgacattggtaaccctaaagctattaagtgtgtacctcaagctgatgtagaatggaagttctatgatgcacagccttgtagtgacaaagcttataaaatagaagaattattctattcttatgccacacattctgacaaattcacagatggtgtatgcctattttggaattgcaatgtcgatagatatcctgctaattccattgtttgtagatttgacactagagtgctatctaaccttaacttgcctggttgtgatggtggcagtttgtatgtaaataaacatgcattccacacaccagcttttgataaaagtgcttttgttaatttaaaacaattaccatttttctattactctgacagtccatgtgagtctcatggaaaacaagtagtgtcagatatagattatgtaccactaaagtctgctacgtgtataacacgttgcaatttaggtggtgctgtctgtagacatcatgctaatgagtacagattgtatctcgatgcttataacatgatgatctcagctggctttagcttgtgggtttacaaacaatttgatacttataacctctggaacacttttacaagacttcagagtttagaaaatgtggcttttaatgttgtaaataagggacactttgatggacaacagggtgaagtaccagtttctatcattaataacactgtttacacaaaagttgatggtgttgatgtagaattgtttgaaaataaaacaacattacctgttaatgtagcatttgagctttgggctaagcgcaacattaaaccagtaccagaggtgaaaatactcaataatttgggtgtggacattgctgctaatactgtgatctgggactacaaaagagatgctccagcacatatatctactattggtgtttgttctatgactgacatagccaagaaaccaactgaaacgatttgtgcaccactcactgtcttttttgatggtagagttgatggtcaagtagacttatttagaaatgcccgtaatggtgttcttattacagaaggtagtgttaaaggtttacaaccatctgtaggtcccaaacaagctagtcttaatggagtcacattaattggagaagccgtaaaaacacagttcaattattataagaaagttgatggtgttgtccagcaattacctgaaacttactttactcagagtagaaatttacaagaatttaaacccaggagtcaaatggaaattgatttcttagaattagctatggatgaattcattgaacggtataaattagaaggctatgccttcgaacatatcatttatggagattttagtcatagtcagttaggtggtttacatctactgattggactagctaaacgttttaaggaatcaccttttgaattagaagattttattcctatggacagtacagttaaaaactatttcataacagatgcgcaaacaggttcatctaagtgtgtgtgttctgttattgatttattacttgatgattttgttgaaataataaaatcccaagatttatctgtagtttctaaggttgtcaaagtgactattgactatacagaaatttcatttatgctttggtgtaaagatggccatgtagaaacattttacccaaaattacaatctagtcaagcatggcaaccaggtgttgctatgcctaatctttacaaaatgcaaagaatgctattagaaaagtgtgaccttcaaaattatggtgatagtgcaacattacctaaaggcataatgatgaatgtcgcaaaatatactcaactgtgtcaatatttaaacacattaacattagctgtaccctataatatgagagttatacattttggtgctggttctgataaaggagttgcaccaggtacagctgttttaagacagtggttgcctacgggtacgctgcttgtcgattcagatcttaatgactttgtctctgatgcagattcaactttgattggtgattgtgcaactgtacatacagctaataaatgggatctcattattagtgatatgtacgaccctaagactaaaaatgttacaaaagaaaatgactctaaagagggttttttcacttacatttgtgggtttatacaacaaaagctagctcttggaggttccgtggctataaagataacagaacattcttggaatgctgatctttataagctcatgggacacttcgcatggtggacagcctttgttactaatgtgaatgcgtcatcatctgaagcatttttaattggatgtaattatcttggcaaaccacgcgaacaaatagatggttacgtaatgcatgcaaattacatattttggaggaatacaaatccaattcagttgtcttcctattctttatttgacatgagtaaatttccccttaaattaaggggtactgctgttatgtctttaaaagaaggtcaaatcaatgatatgattttatctcttcttagtaaaggtagacttataattagagaaaacaacagagttgttatttctagtgatgttcttgttaacaactaaacgaacaatgtttgtttttcttgttttattgccactagtctctagtcagtgtgttaatcttacaaccagaactcaattaccccctgcatacactaattctttcacacgtggtgtttattaccctgacaaagttttcagatcctcagttttacattcaactcaggacttgttcttacctttcttttccaatgttacttggttccatgctatacatgtctctgggaccaatggtactaagaggtttgataaccctgtcctaccatttaatgatggtgtttattttgcttccactgagaagtctaacataataagaggctggatttttggtactactttagattcgaagacccagtccctacttattgttaataacgctactaatgttgttattaaagtctgtgaatttcaattttgtaatgatccatttttgggtgtttattaccacaaaaacaacaaaagttggatggaaagtgagttcagagtttattctagtgcgaataattgcacttttgaatatgtctctcagccttttcttatggaccttgaaggaaaacagggtaatttcaaaaatcttagggaatttgtgtttaagaatattgatggttattttaaaatatattctaagcacacgcctattaatttagtgcgtgatctccctcaggggttttcggctttagaaccattggtagatttgccaataggtattaacatcactaggtttcaaactttacttgctttacatagaagttatttgactcctggtgattcttcttcaggttggacagctggtgctgcagcttattatgtgggttatcttcaacctaggacttttctattaaaatataatgaaaatggaaccattacagttgctgtagcctgtgcacttgaccctctctcagaaacaaagtgtacgttgaaatccttcactgtagaaaaaggaatctatcaaacttctaactttagagtccaaccaacagaatctattgttagatttcctaatattacaaacttgtgcccttttggtgaagtttttaacgccaccagatttgcatctgtttatgcttggaacaggaagagaatcagcaactgtgttgctgattattctgtcctatataattccgcatcattttccacttttaagtgttatggagtgtctcctactaaattaaatgatctctgctttactaatgtctatgcagattcatttgtaattagaggtgatgaagtcagacaaatcgctccagggcaaactggaaagattgctgattataattataaattaccagatgattttacaggctgcgttatagcttggaattctaacaatcttgattctaaggttggtggtaattataattacctgtatagattgtttaggaagtctaatctcaaaccttttgagagagatatttcaactgaaatctatcaggccggtagcacaccttgtaatggtgttgaaggttttaattgttactttcctttacaatcatatggtttccaacccactaatggtgttggttaccaaccatacagagtagtagtactttcttttgaacttctacatgcaccagcaactgtttgtggacctaaaaagtctactaatttggttaaaaacaaatgtgtcaatttcaacttcaatggtttaacaggcacaggtgttcttactgagtctaacaaaaagtttctgcctttccaacaatttggcagagacattgctgacactactgatgctgtccgtgatccacagacacttgagattcttgacattacaccatgttcttttggtggtgtcagtgttataacaccaggagcaaatacatctaaccaagttactgttctttatcaggatgttaactgcacagaagtccctgttgctattcatgcagatcaacttactcctacttggcgtgtttattctacaggttctaatgttttcaaaacacgtgcaggctgtttaataggggctgaacatgtcaacaactcatatgagtgtgacatacccattggtgcaggtatatgcgctagttatcaaactcagactaattctcctcggcgggcacgaagtacagctagtcaatccatcattgcctacactatgtcacttggtgcagaaaattcagttgcttactctaacaactctattgtcatacccacaaattttactattagtgttaccacagaaattctaccagtgtctatgaccaagacatcagtagattgtacaatgtacatttgtagtgattcaactgaatgcagcaatcctttgttacaatatggcagtttttgcacacaattaaaccgtgctttaactggaatagctgttgaacaagacaaaaacacccaagaagtttttgcacaagtcaaacaaatttacaaaacaccaccaattaaagattttggtggttttaatttttcacaaatattaccagatccatcaaaaccaagcaagaggtcatttattgaagatctacttttcaacaaagtgacacttgcagatgctggcttcatcaaacaatatggtgattgccttggtgatattgctgctagagacctcatttgtgcacaaaagtttaacggccttactgttttgccacctttgctcacagatgaaatgattgctcaatacacttctgcactgttagcgggtacaatcacttctggttggacctttggtgcaggtgctgcattacaaataccatttgctatgcaaatggcttataggtttaatggtattagagttacacagaatgttctctatgagaaccaaaaattgattgccaaccaatttaatagtgctattggcaaaattcaagactcactttcttccacagcaagtgcacttggaaaacttcaagatgtggtcaaccaaaatgcacaagctttaaacacgcttgttaaacaacttagctccactttcagcacaatttcaagtgttttaaatgatatcctttcacgtcttgacaaagttgaggctgaagtgcaaattgataggttgatcacaggcagacttcaaagtttgcagacatatgtgactcaacaattaattagagctgcagaaatcagagcttctgctaatcttaaggctactaaaatgtcagagtgtgtacttggacaatcaaaaagagttgatttttgtggaaagggctatcatcttatgtccttccctcagtcagcacctcatggtgtagtcttcttgcatgtgacttatgtccctgcacaagaaaagaacttcacaactgctcctgccacttgtcatgatggaaaagcacactttcctcgtgaaggtgtctttgtttcaaatggcacacactggtttgtaacacaaaggaattttgatgaaccacaaatcattactacagacaacacatttgtgtctggtaactgtgatgttgtaataggaattgtcaacaacacagtttatgatcctttgcaacctgaattagactcattcaaggaggagttagataaatattttaagaatcatacatcaccagatgttgatttaggtgacatctctggcattaatgcttcagttgtaaacattcaaaaagaaattgaccgcctcaatgaggttgccaagaatttaaatgaatctctcatcgatctccaagaacttggaaagtatgagcagtatataaaatggccatggtacatttggctaggttttatagctggcttgattgccatagtaatggtgacaattatgctttgctgtatgaccagttgctgtagttgtctcaagggctgttgttcttgtggatcctgctgcaaatttgatgaagacgactctgagccagtgctcaaaggagtcaaattacattacacataaacgaacttatggatttgtttatgagaatcttcacaattggaactgtaactttgaagcaaggtgaaatcaaggatgctactccttcagattttgttcgcgctactgcaacgataccgatacaagcctcactccctttcggatggcttattgttggcgttgcacttcttgctgtttttcagagcgcttccaaaatcataaccctcaaaaagagatggcaactagcactctccaagggtgttcactttgtttgcaacttgctgttgttgtttgtaacagtttactcacaccttttgctcgttgctgctggcttgtaagccccttttctctatctttatgctttagtctacttcttgcagagtataaactttgtaagaataataatgaggctttggctttgctggaaatgccgttccaaaaacccattactttatgatgccaactattttctttgctggcatactaattgttatgactattgtataccttacaatagtgtaacttcttcaattgtcattacttcaggtgatggcacaacaagtcctatttctgaacatgactaccagattggtggttatactgaaaaatgggaatctggagtaaaagactgtgttgtattacacagttacttcacttcagactattaccagctgtactcaactcaattgagtacagacactggtgttgaacatgttaccttcttcatctacaataaaattgttgatgagcctgaagaacatgtccaaattcacacaatcgacggttcatccggagttgttaatccagtaatggaaccaatttatgatgaaccgacgacgactactagcgtgcctttgtaatgcacaagctgatgagtacgaacttatgtactcattcgtttcggaagagacaggtacgttaatagttaatagcgtacttctttttcttgctttcgtggtattcttgctagttacactagccatccttactgcgcttcgattgtgtgcgtactgctgcaatattgttaacgtgagtcttgtaaaaccttctttttacgtttactctcgtgttaaaaatctgaattcttctagagttcctgatcttctggtctaaacgaactaaatattatattagtttttctgtttggaactttaattttagccatggcagattccaacggtactattaccgttgaagagcttaaaaagctccttgaacaatggaacctagtaataggtttcctattccttacatggatttgtcttctacaatttgcctatgccaacaggaataggtttttgtatataattaagttaattttcctctggctgttatggccagtaactttagcttgttttgtgcttgctgctgtttacagaataaattggatcaccggtggaattgctatcgcaatggcttgtcttgtaggcttgatgtggctcagctacttcattgcttctttcagactgtttgcgcgtacgcgttccatgtggtcattcaatccagaaactaacattcttctcaacgtgccactccatggcactattctgaccagaccgcttctagaaagtgaactcgtaatcggagctgtgatccttcgtggacatcttcgtattgctggacaccatctaggacgctgtgacatcaaggacctgcctaaagaaatcactgttgctacatcacgaacgctttcttattacaaattgggagcttcgcagcgtgtagcaggtgactcaggttttgctgcatacagtcgctacaggattggcaactataaattaaacacagaccattccagtagcagtgacaatattgctttgcttgtacagtaagtgacaacagatgtttcatctcgttgactttcaggttactatagcagagatattactaattattatgaggacttttaaagtttccatttggaatcttgattacatcataaacctcataattaaaaatttatctaagtcactaactgagaataaatattctcaattagatgaagagcaaccaatggagattgattaaacgaacatgaaaattattcttttcttggcactgataacactcgctacttgtgagctttatcactaccaagagtgtgttagaggtacaacagtacttttaaaagaaccttgctcttctggaacatacgagggcaattcaccatttcatcctctagctgataacaaatttgcactgacttgctttagcactcaatttgcttttgcttgtcctgacggcgtaaaacacgtctatcagttacgtgccagatcagtttcacctaaactgttcatcagacaagaggaagttcaagaactttactctccaatttttcttattgttgcggcaatagtgtttataacactttgcttcacactcaaaagaaagacagaatgattgaactttcattaattgacttctatttgtgctttttagcctttctgctattccttgttttaattatgcttattatcttttggttctcacttgaactgcaagatcataatgaaacttgtcacgcctaaacgaacatgaaatttcttgttttcttaggaatcatcacaactgtagctgcatttcaccaagaatgtagtttacagtcatgtacgcaatatcaaccacatgtagttgatgacccgtgtcctattcacttctattctaaatggtatattagagtaggagctagaaaatcagcacctttaattgaattgtgcgtggatgaggctggttctaaatcacccattcagtacatcgatatcggtaattatacagtttcctgtttaccttttacaattaattgccaggaacctaaattgggtagtcttgtagtgcgttgttcgttctatgaagactttttagagtatcatgacgttcgtgttgttttagatttcatctaaacgaacaaactaaaatgtctgataatggaccccaaaatcagcgaaatgcaccccgcattgcttttggtggaccctcagattcaactggcagtaaccagaatggagaacgcagtggggcgcgatcaaaacaacgtcggccccaaggtttacccaataatactgcgtcttggttcaccgctctcactcaacatggcaaggaagaccttaaattccctcgaggacaaggcgttccaattaacaccaatagcagtccagatgaccaaattggctactaccgaagagctaccagacgaattcgtggtggtgacggtaaaatgaaagatctcagtccaagatggtatttctactacctaggaactgggccagaagctggacttccctatggtgctaacaaagacggcatcatatgggttgcaactgagggagccttgaatacaccaaaagatcacattggcacccgcaatcctgctaacaatgctgcaatcgtgctacaacttcctcaaggaacaacattgccaaaaggcttctacgcagaagggagcagaggcggcagtcaagcctcttctcgttcctcatcacgtagtcgcaacagttcaagaaattcaactccaggcagcagtaggggaacttctcctgctagaatggctggcaatggcggtgatgctgctcttgctttgctgctgcttgacagattgaaccagcttgagagcaaaatgtctggtaaaggccaacaacaacaaggccaaactgtcactaagaaatctgctgctgaggcttctaagaagcctcggcaaaaacgtactgccactaaagcatacaatgtaacacaagctttcggcagacgtggtccagaacaaacccaaggaaattttggggaccaggaactaatcagacaaggaactgattacaaacattggccgcaaattgcacaatttgcccccagcgcttcagcgttcttcggaatgtcgcgcattggcatggaagtcacaccttcgggaacgtggttgacctacacaggtgccatcaaattggatgacaaagatccaaatttcaaagatcaagtcattttgctgaataagcatattgacgcatacaaaacattcccaccaacagagcctaaaaaggacaaaaagaagaaggctgatgaaactcaagccttaccgcagagacagaagaaacagcaaactgtgactcttcttcctgctgcagatttggatgatttctccaaacaattgcaacaatccatgagcagtgctgactcaactcaggcctaaactcatgcagaccacacaaggcagatgggcaatacaaacgttttcgcttttccgtttacgatatatagtctactcttgtgcagaatgaattctcgtaactacatagcacaagtagatgtagttaactttaatctcacatagcaatctttaatcagtgtgtaacattagggaggacttgaaagagccaccacattttcaccgaggccacgcggagtacgatcgagtgtacagtgaacaatgctagggagagctgcctatatggaagagccctaatg

SEQ ID NO: 20 - DNA, 21 bp, artificial sequence
  synthetic oligonucleotide (FW-primer MUT-As)
gctagttgggtgatgcgtatt

SEQ ID NO: 21 - DNA, 22 bp, artificial sequence
  synthetic oligonucleotide (FW primer MUT-Bs)
tggtctatatgcctgctagttg

SEQ ID NO: 22 - DNA, 23 bp, artificial sequence
  synthetic oligonucleotide (FW primer MUT-Cs)
gatgcgtattatgacatggttgg

SEQ ID NO: 23 - DNA, 22 bp, artificial sequence
  synthetic oligonucleotide (FW primer MUT-Ds)
tctcttgccactgtagcttatt

SEQ ID NO: 24 - DNA, 23 bp, artificial sequence
  synthetic oligonucleotide (FW primer MUT-Fs)
gtgatgcgtattatgacatggtt

SEQ ID NO: 25 - DNA, 23 bp, artificial sequence
  synthetic oligonucleotide (RV primer MUT-Ar)
ctcctagcaccatcatcatacac

SEQ ID NO: 26 - DNA, 23 bp, artificial sequence
  synthetic oligonucleotide (RV primer MUT-Br)
gctgatgcatacataacacagtc

SEQ ID NO: 27 - DNA, 25 bp, artificial sequence
  synthetic oligonucleotide (RV primer MUT-Cr)
cagttcttgctgtcataaggattag

SEQ ID NO: 28 - DNA, 24 bp, artificial sequence
  synthetic oligonucletide (RV primer MUT-Dr)
gattagtaacactacagctgatgc

SEQ ID NO: 29 - DNA, 22 bp, artificial sequence
  synthetic oligonucleotide (MUT-probe A (FW))
tggttgatactagtttgaagct

SEQ ID NO: 30 - DNA, 26 bp, artificial sequence
  synthetic oligonucleotide (MUT-probeB (RV))
gcttcaaactagtatcaaccatatcc

SEQ ID NO: 31 - DNA, 21 bp, artificial sequence
  synthetic oligonucleotide (FW primer UK-As)
agtgcgttgttcgttctatga

SEQ ID NO: 32 - DNA, 22 bp, artificial sequence
  synthetic oligonucleotide (FW primer UK-Bs)
agtatcatgacgttcgtgttgt

SEQ ID NO: 33 - DNA, 24 bp, artificial sequence
  synthetic oligonucleotide (FW primer UK-Cs)
cgttgttcgttctatgaagacttt

SEQ ID NO: 34 - DNA, 21 bp, artificial sequence
  synthetic oligonucleotide  (FW primer UK-Ds)
tcatgacgttcgtgttgtttt

SEQ ID NO: 35 - DNA, 21 bp, artificial sequence
  synthetic oligonucleotide (FW primer UK-D2s)
tgcgttgttcgttctatgaag

SEQ ID NO: 36 - DNA, 20 bp, artificial sequence
  synthetic oligonucleotide (FW primer UK-Es)
ttctccattctggttactgc

SEQ ID NO: 37 - DNA, 20 bp, artificial sequence
  synthetic oligonucleotide (FW primer UK-Fs)
tgacgttcgtgttgttttag

SEQ ID NO: 38 - DNA, 20 bp, artificial sequence
  synthetic oligonucleotide (RV primer UK-Ar)
agggtccaccaaacgtaatg

SEQ ID NO: 39 - DNA, 21 bp, artificial sequence
  synthetic oligonucleotide (RV primer UK-Br)
gcgttctccattctggttact

SEQ ID NO: 40 - DNA, 20 bp, artificial sequence
  synthetic oligonucleotide (RV primer UK-Cr)
gaatctgagggtccaccaaa

SEQ ID NO: 41 - DNA, 20 bp, artificial sequence
  synthetic oligonucleotide (RV primer UK-Dr)
ctgcgttctccattctggtt

SEQ ID NO: 42 - DNA, 20 bp, artificial sequence
  synthetic oligonucleotide (RV primer UK-Er)
gtagtgcgttgttcgttcta

SEQ ID NO: 43 - DNA, 20 bp, artificial sequence
  synthetic oligonucleotide (RV primer UK-Fr)
ctggttactgccagttgaat

SEQ ID NO: 44 - DNA, 27 bp, artificial sequence
  synthetic oligonucleotide (UK-probeA FW)
tgtctctaaatggaccccaaaatcagc

SEQ ID NO: 45 - DNA, 24 bp, artificial sequence
  synthetic oligonucleotide (UK-probeB RV)
gctgattttggggtccatttagag

SEQ ID NO: 46 - DNA, 24 bp, artificial sequence
  synthetic oligonucleotide (UK-probeC FW)
ctctaaatggaccccaaaatcagc